European Patent Application EP 4 741 500 A1, published May 13, 2026. Title: Polynucleotide, Pharmaceutical Composition and Uses Thereof. Applicant: LIANGZHU LABORATORY. Application WO PCT/CN2024/098005, filed June 7, 2024. The sequence listing filed with the application follows.

SEQUENCE LISTING (11 sequences)

SEQ ID NO: 1 - DNA, 29 bp, synthetic construct
  source 1..29: mol_type = other DNA
cacatctgccttaaaaccaaagagggctt

SEQ ID NO: 2 - DNA, 20 bp, synthetic construct
  source 1..20: mol_type = other DNA
ttggttttaaggcagatgtg

SEQ ID NO: 3 - DNA, 20 bp, synthetic construct
  source 1..20: mol_type = other DNA
ctttggttttaaggcagatg

SEQ ID NO: 4 - DNA, 20 bp, synthetic construct
  source 1..20: mol_type = other DNA
ctctttggttttaaggcaga

SEQ ID NO: 5 - DNA, 20 bp, synthetic construct
  source 1..20: mol_type = other DNA
cctctttggttttaaggcag

SEQ ID NO: 6 - DNA, 20 bp, synthetic construct
  source 1..20: mol_type = other DNA
ccctctttggttttaaggca

SEQ ID NO: 7 - DNA, 20 bp, synthetic construct
  source 1..20: mol_type = other DNA
gccctctttggttttaaggc

SEQ ID NO: 8 - DNA, 20 bp, synthetic construct
  source 1..20: mol_type = other DNA
agccctctttggttttaagg

SEQ ID NO: 9 - DNA, 20 bp, synthetic construct
  source 1..20: mol_type = other DNA
aagccctctttggttttaag

SEQ ID NO: 10 - DNA, 25 bp, synthetic construct
  source 1..25: mol_type = other DNA
catctgccttaaaaccaaagagggc

SEQ ID NO: 11 - DNA, 981 bp, synthetic construct
  source 1..981: mol_type = other DNA
atctgggacctgccaggcaggggtgggggtggaggcttcctgcgtcctcctcacctcatgcccaccccctgccctgcacgtcatgggagggggcttgaagccaaagaaaaataaccctttggtttttttcttctgtatttttttttctaagagaagttattttctacagtggttttatactgaaggaaaaacacaagcaaaaaaaaaaaaaagcatctatctcatctatctcaatcctaatttctcctcccttccttttccctgcttccaggaaactccacatctgccttaaaaccaaagagggcttcctctagaagccaagggaaaggggtgcttttatagaggctagcttctgcttttctgccctggctgctgcccccaccccggggaccctgtgacatggtgcctgagaggcaggcatagaggcttctccgccagcctcctctggacggcaggctcactgccaggccagcctccgagagggagagagagagagagaggacagcttgagccgggcccctgggcttggcctgctgtgattccactacacctggctgaggttcctctgcctgccccgcccccagtccccacccctgcccccagccccggggtgagtccattctcccaggtaccagctgcgcttgcttttctgtattttatttagacaagagatgggaatgaggtgggaggtggaagaagggagaagaaaggtgagtttgagctgccttccctagctttagaccctgggtgggctctgtgcagtcactggaggttgaagccaagtggggtgctgggaggagggagagggaggtcactggaaaggggagagcctgctggcacccaccgtggaggaggaaggcaagagggggtggaggggtgtggcagtggttttggcaaacgctaaagagcccttgcctccccatttcccatctgcaccccttctctcctccccaaatcaatacactagttgtttctacccct